European Patent Application EP 4 800 035 A1, published September 2, 2026. Title: Antibody against interleukin-7 receptor (IL-7R) and antibody-drug conjugate (ADC) comprising the same. Applicant: National Cancer Center. The sequence listing filed with the application follows.

SEQUENCE LISTING (66 sequences)

SEQ ID NO: 1 - DNA, 45 bp, synthetic construct
  source 1..45: mol_type = other DNA
ctaatacgactcactatagggcaagcagtggtatcaacgcagagt

SEQ ID NO: 2 - DNA, 28 bp, synthetic construct
  source 1..28: mol_type = other DNA
ggactctgggatcatttacccggagagt

SEQ ID NO: 3 - DNA, 27 bp, synthetic construct
  source 1..27: mol_type = other DNA
ccttaggagggaagattggaaggagct

SEQ ID NO: 4 - protein, 330 aa, Homo sapiens
ASTKGPSVFPLAPSSKSTSGGTAALGCLVKDYFPEPVTVSWNSGALTSGVHTFPAVLQSSGLYSLSSVVTVPSSSLGTQTYICNVNHKPSNTKVDKKVEPKSCDKTHTCPPCPAPELLGGPSVFLFPPKPKDTLMISRTPEVTCVVVDVSHEDPEVKFNWYVDGVEVHNAKTKPREEQYNSTYRVVSVLTVLHQDWLNGKEYKCKVSNKALPAPIEKTISKAKGQPREPQVYTLPPSREEMTKNQVSLTCLVKGFYPSDIAVEWESNGQPENNYKTTPPVLDSDGSFFLYSKLTVDKSRWQQGNVFSCSVMHEALHNHYTQKSLSLSPGK

SEQ ID NO: 5 - protein, 327 aa, Homo sapiens
ASTKGPSVFPLAPCSRSTSESTAALGCLVKDYFPEPVTVSWNSGALTSGVHTFPAVLQSSGLYSLSSVVTVPSSSLGTKTYTCNVDHKPSNTKVDKRVESKYGPPCPPCPAPEFLGGPSVFLFPPKPKDTLMISRTPEVTCVVVDVSQEDPEVQFNWYVDGVEVHNAKTKPREEQFNSTYRVVSVLTVLHQDWLNGKEYKCKVSNKGLPSSIEKTISKAKGQPREPQVYTLPPSQEEMTKNQVSLTCLVKGFYPSDIAVEWESNGQPENNYKTTPPVLDSDGSFFLYSRLTVDKSRWQEGNVFSCSVMHEALHNHYTQKSLSLSLGK

SEQ ID NO: 6 - protein, 109 aa, synthetic construct
LRRTVAAPSVFIFPPSDEQLKSGTASVVCLLNNFYPREAKVQWKVDNALQSGNSQESVTEQDSKDSTYSLSSTLTLSKADYEKHKVYACEVTHQGLSSPVTKSFNRGEC

SEQ ID NO: 7 - protein, 30 aa, Homo sp.
EVQLVESGGGLVQPGGSLRLSCAASGFNIK

SEQ ID NO: 8 - protein, 14 aa, Homo sapiens
WVRQAPGKGLEWVA

SEQ ID NO: 9 - protein, 32 aa, Homo sapiens
RFTISADTSKNTAYLQMNSLRAEDTAVYYCSR

SEQ ID NO: 10 - protein, 11 aa, Homo sapiens
WGQGTLVTVSS

SEQ ID NO: 11 - protein, 23 aa, Homo sapiens
DIQMTQSPSSLSASVGDRVTITC

SEQ ID NO: 12 - protein, 15 aa, Homo sapiens
WYQQKPGKAPKLLIY

SEQ ID NO: 13 - protein, 32 aa, Homo sapiens
GVPSRFSGSRSGTDFTLTISSLQPEDFATYYC

SEQ ID NO: 14 - protein, 8 aa, Homo sapiens
FGQGTKVE

SEQ ID NO: 15 - protein, 117 aa, synthetic construct
EVQLQQSGAELVKPGASVKLSCTVSGFNIKDTYIHWVKQRPEQGLEWIGRIDPASDDTKYDPKFQGKATLTADTSSNTAYLQLSSLTSEDTAVYYCVRRVYDYLDYWGQGTTLTVSS

SEQ ID NO: 16 - protein, 105 aa, synthetic construct
ETTVTQSPASLSMAMGEKVTIRCMTSTDINDDMNWYQQKPGEPPKLLISEGNTLRPGVPSRFSSSGYSTDFFFTIEYMLSEDVADYFCLQTDNLPLTFGAGTKLE

SEQ ID NO: 17 - protein, 5 aa, synthetic construct
DTYIH

SEQ ID NO: 18 - protein, 17 aa, synthetic construct
RIDPASDDTKYDPKFQG

SEQ ID NO: 19 - protein, 8 aa, synthetic construct
RVYDYLDY

SEQ ID NO: 20 - protein, 11 aa, synthetic construct
MTSTDINDDMN

SEQ ID NO: 21 - protein, 7 aa, synthetic construct
EGNTLRP

SEQ ID NO: 22 - protein, 9 aa, synthetic construct
LQTDNLPLT

SEQ ID NO: 23 - protein, 114 aa, synthetic construct
QVQLQQSGAELVKPGASVKLSCKASGYTFTNYYMYWVKQRPGQGLEWIGEINPSNGGTNFNEKFKSKATLTVDKSSSTAYMQLSSLTSEDSAVYYCTRRSFAYWGQGTLVTVSA

SEQ ID NO: 24 - protein, 105 aa, synthetic construct
DIVMTQSHKFMSTSVGDRVSITCKASQDVGIVVAWYQQKPGQSPKLLIYWASTRHTGVPDRFTGSGSGTDFTLTISNVQSEDLADYFCQQYSSYPLTFGAGTKLE

SEQ ID NO: 25 - protein, 5 aa, synthetic construct
NYYMY

SEQ ID NO: 26 - protein, 17 aa, synthetic construct
EINPSNGGTNFNEKFKS

SEQ ID NO: 27 - protein, 5 aa, synthetic construct
RSFAY

SEQ ID NO: 28 - protein, 11 aa, synthetic construct
KASQDVGIVVA

SEQ ID NO: 29 - protein, 7 aa, synthetic construct
WASTRHT

SEQ ID NO: 30 - protein, 9 aa, synthetic construct
QQYSSYPLT

SEQ ID NO: 31 - protein, 115 aa, synthetic construct
EVQLQQSGPELEKPGASVKISCKASGYSFTGYNMNWVKQSNGESLEWIGIIDPYSGDTTYNQKFKGKATLTVDKSSSTAYMQLKSLTSDDSAVYYCTRLDWEAYWGQGTLVTVSA

SEQ ID NO: 32 - protein, 104 aa, synthetic construct
QIVLTQSPAIMSSFPGEKVTMTCSASSSVNYIHWYQQKSGTSPKRLIYDTSKLASGVPPRFSGSGSGTSYSLTISSMEAEDAATYYCQQWSRNPLTFGAGTKLE

SEQ ID NO: 33 - protein, 5 aa, synthetic construct
GYNMN

SEQ ID NO: 34 - protein, 17 aa, synthetic construct
IIDPYSGDTTYNQKFKG

SEQ ID NO: 35 - protein, 6 aa, synthetic construct
LDWEAY

SEQ ID NO: 36 - protein, 10 aa, synthetic construct
SASSSVNYIH

SEQ ID NO: 37 - protein, 7 aa, synthetic construct
DTSKLAS

SEQ ID NO: 38 - protein, 9 aa, synthetic construct
QQWSRNPLT

SEQ ID NO: 39 - protein, 118 aa, synthetic construct
EVQLQQSGPELVKPGTSVKISCKTSGSTFTEYTMHWVKQSHGKSLEWIGGFNPDNGGTTYNQKFKGKATLTVDKSSSTAHMELRSLTSDDSAVYYCTRDYGFVRFVYWGQGTLVTVSA

SEQ ID NO: 40 - protein, 105 aa, synthetic construct
DIQMTQTTSSLSASLGDRVTISCRTSQDISNYLNWYQQKPDGTVKLLIYYTSRLHSGVPSRFSGSGSGTDYSLTISNLEQEDIATYFCQQGNTLPYTFGGGTKLE

SEQ ID NO: 41 - protein, 5 aa, synthetic construct
EYTMH

SEQ ID NO: 42 - protein, 17 aa, synthetic construct
GFNPDNGGTTYNQKFKG

SEQ ID NO: 43 - protein, 9 aa, synthetic construct
DYGFVRFVY

SEQ ID NO: 44 - protein, 11 aa, synthetic construct
RTSQDISNYLN

SEQ ID NO: 45 - protein, 7 aa, synthetic construct
YTSRLHS

SEQ ID NO: 46 - protein, 9 aa, synthetic construct
QQGNTLPYT

SEQ ID NO: 47 - protein, 117 aa, synthetic construct
EVQLVQSGAEVKKPGASVKVSCTVSGYTIKDTYIHWVKQAPEQGLEWMGRIDPASDDTKYDPKFQGKVTLTADTSINTAYLQLSSLTSEDTAVYYCVRRVYDYLDYWGQGTTVTVSS

SEQ ID NO: 48 - protein, 105 aa, synthetic construct
ETTLTQSPAFMSATMGDKVTISCMTSTDINDDMNWYQQKPGEPPILIIQEGNTLRPGIPPRFSGSGYGTDFTFTINNMLSEDAADYFCLQTDNLPLTFGGGTKLE

SEQ ID NO: 49 - protein, 118 aa, synthetic construct
EVQLVQSGAEVKKPGASVKVSCKVSGYTFTEYTMHWVKQAPGKGLEWMGGFNPDNGGTTYNQKFKGKVTLTVDTSTSTAYMELRSLRSEDTAVYYCARDYGFVRFVYWGQGTLVTVSA

SEQ ID NO: 50 - protein, 105 aa, synthetic construct
DIQMTQSPSSLSASLGDRVTITCRTSQDISNYLNWYQQKPGEAVILIIQYTSRLHSGVPSRFSGSGSGTDYTFTISNLQQEDIATYYCQQGNTLPYTFGGGTKVE

SEQ ID NO: 51 - protein, 30 aa, synthetic construct
EVQLVQSGAEVKKPGASVKVSCTVSGYTIK

SEQ ID NO: 52 - protein, 14 aa, synthetic construct
WVKQAPEQGLEWMG

SEQ ID NO: 53 - protein, 32 aa, synthetic construct
KVTLTADTSINTAYLQLSSLTSEDTAVYYCVR

SEQ ID NO: 54 - protein, 11 aa, synthetic construct
WGQGTTVTVSS

SEQ ID NO: 55 - protein, 23 aa, synthetic construct
ETTLTQSPAFMSATMGDKVTISC

SEQ ID NO: 56 - protein, 15 aa, synthetic construct
WYQQKPGEPPILIIQ

SEQ ID NO: 57 - protein, 32 aa, synthetic construct
GIPPRFSGSGYGTDFTFTINNMLSEDAADYFC

SEQ ID NO: 58 - protein, 8 aa, synthetic construct
FGGGTKLE

SEQ ID NO: 59 - protein, 30 aa, synthetic construct
EVQLVQSGAEVKKPGASVKVSCKVSGYTFT

SEQ ID NO: 60 - protein, 14 aa, synthetic construct
WVKQAPGKGLEWMG

SEQ ID NO: 61 - protein, 32 aa, unidentified
KVTLTVDTSTSTAYMELRSLRSEDTAVYYCAR

SEQ ID NO: 62 - protein, 11 aa, synthetic construct
WGQGTLVTVSA

SEQ ID NO: 63 - protein, 23 aa, synthetic construct
DIQMTQSPSSLSASLGDRVTITC

SEQ ID NO: 64 - protein, 15 aa, synthetic construct
WYQQKPGEAVILIIQ

SEQ ID NO: 65 - protein, 32 aa, synthetic construct
GVPSRFSGSGSGTDYTFTISNLQQEDIATYYC

SEQ ID NO: 66 - protein, 8 aa, synthetic construct
FGGGTKVE